European Patent Application EP 4 538 293 A1, published April 16, 2025. Title: CD39/CD73 BISPECIFIC ANTIGEN BINDING PROTEIN AND USE THEREOF TECHNICAL FIELD. Applicant: 上海华奥泰生物药业股份有限公司. The sequence listing filed with the application follows.

SEQUENCE LISTING (49 sequences)

SEQ ID NO: 1 - protein, 18 aa, synthetic construct
  REGION 1..18: note = 700053 CDR3
NAWGEDDSSWFGTDLCDY

SEQ ID NO: 2 - protein, 7 aa, synthetic construct
  REGION 1..7: note = 700053 CDR2
ITSGGNT

SEQ ID NO: 3 - protein, 8 aa, synthetic construct
  REGION 1..8: note = 700053 CDR1
GSISSIAA

SEQ ID NO: 4 - protein, 25 aa, synthetic construct
  REGION 1..25: note = 700053 FR1
QVQLVESGGGLVQPGGSLRLSCAAS

SEQ ID NO: 5 - protein, 17 aa, synthetic construct
  REGION 1..17: note = 700053 FR2
MGWYRQAPGKERELVAA

SEQ ID NO: 6 - protein, 38 aa, synthetic construct
  REGION 1..38: note = 700053 FR3
NLADSTKGRFTISRDNTKNTVYLQMNSLKPEDTAVYYC

SEQ ID NO: 7 - protein, 11 aa, synthetic construct
  REGION 1..11: note = 700053 FR4
WGQGTQVTVSS

SEQ ID NO: 8 - protein, 124 aa, synthetic construct
  REGION 1..124: note = 700053 VHH
QVQLVESGGGLVQPGGSLRLSCAASGSISSIAAMGWYRQAPGKERELVAAITSGGNTNLADSTKGRFTISRDNTKNTVYLQMNSLKPEDTAVYYCNAWGEDDSSWFGTDLCDYWGQGTQVTVSS

SEQ ID NO: 9 - protein, 18 aa, synthetic construct
  REGION 1..18: note = 900698 HCDR3
ARAIYYYGSSYNYYAMDY

SEQ ID NO: 10 - protein, 8 aa, synthetic construct
  REGION 1..8: note = 900698 HCDR2
ISSGGGYI

SEQ ID NO: 11 - protein, 8 aa, synthetic construct
  REGION 1..8: note = 900698 HCDR1
GFTFSKYA

SEQ ID NO: 12 - protein, 25 aa, synthetic construct
  REGION 1..25: note = 900698 H-FR1
QVQLVESGGGLVKPGGSLRLSCAAS

SEQ ID NO: 13 - protein, 17 aa, synthetic construct
  REGION 1..17: note = 900698 H-FR2
MSWIRQAPGKGLEWVAE

SEQ ID NO: 14 - protein, 38 aa, synthetic construct
  REGION 1..38: note = 900698 H-FR3
NYADSVKGRFTISRDNAKNSLYLQMNSLRAEDTAVYYC

SEQ ID NO: 15 - protein, 11 aa, synthetic construct
  REGION 1..11: note = 900698/90725 H-FR4
WGQGTTVTVSS

SEQ ID NO: 16 - protein, 125 aa, synthetic construct
  REGION 1..125: note = 900698 VH
QVQLVESGGGLVKPGGSLRLSCAASGFTFSKYAMSWIRQAPGKGLEWVAEISSGGGYINYADSVKGRFTISRDNAKNSLYLQMNSLRAEDTAVYYCARAIYYYGSSYNYYAMDYWGQGTTVTVSS

SEQ ID NO: 17 - protein, 9 aa, synthetic construct
  REGION 1..9: note = 900698 LCDR3
QQYSSYPLT

SEQ ID NO: 18 - skipped

SEQ ID NO: 19 - protein, 6 aa, synthetic construct
  REGION 1..6: note = 900698 LCDR1
QDVGTA

SEQ ID NO: 20 - protein, 26 aa, synthetic construct [sequence omitted]

SEQ ID NO: 21 - protein, 17 aa, synthetic construct
  REGION 1..17: note = 900698 L-FR2
EAWYQQKPGKAPKLLIY

SEQ ID NO: 22 - protein, 36 aa, synthetic construct
  REGION 1..36: note = 900698 L-FR3
TRHTGVPSRFSGSGSGTDFTLTISSLQPEDFATYYC

SEQ ID NO: 23 - protein, 10 aa, synthetic construct
  REGION 1..10: note = 900698/900725 L-FR4
FGQGTKLEIK

SEQ ID NO: 24 - protein, 107 aa, synthetic construct
  REGION 1..107: note = 900698 VL
DIQMTQSPSSLSASVGDRVTITCRASQDVGTAEAWYQQKPGKAPKLLIYWASTRHTGVPSRFSGSGSGTDFTLTISSLQPEDFATYYCQQYSSYPLTFGQGTKLEIK

SEQ ID NO: 25 - protein, 454 aa, synthetic construct
  REGION 1..454: note = 900698 heavy chain
QVQLVESGGGLVKPGGSLRLSCAASGFTFSKYAMSWIRQAPGKGLEWVAEISSGGGYINYADSVKGRFTISRDNAKNSLYLQMNSLRAEDTAVYYCARAIYYYGSSYNYYAMDYWGQGTTVTVSSASTKGPSVFPLAPSSKSTSGGTAALGCLVKDYFPEPVTVSWNSGALTSGVHTFPAVLQSSGLYSLSSVVTVPSSSLGTQTYICNVNHKPSNTKVDKRVEPKSCDKTHTCPPCPAPEAAGGPSVFLFPPKPKDTLMISRTPEVTCVVVDVSHEDPEVKFNWYVDGVEVHNAKTKPREEQYNSTYRVVSVLTVLHQDWLNGKEYKCKVSNKALPAPIEKTISKAKGQPREPQVYTLPPSREEMTKNQVSLTCLVKGFYPSDIAVEWESNGQPENNYKTTPPVLDSDGSFFLYSKLTVDKSRWQQGNVFSCSVMHEALHNHYTQKSLSLSPG

SEQ ID NO: 26 - protein, 214 aa, synthetic construct
  REGION 1..214: note = 900698 light chain
DIQMTQSPSSLSASVGDRVTITCRASQDVGTAEAWYQQKPGKAPKLLIYWASTRHTGVPSRFSGSGSGTDFTLTISSLQPEDFATYYCQQYSSYPLTFGQGTKLEIKRTVAAPSVFIFPPSDEQLKSGTASVVCLLNNFYPREAKVQWKVDNALQSGNSQESVTEQDSKDSTYSLSSTLTLSKADYEKHKVYACEVTHQGLSSPVTKSFNRGEC

SEQ ID NO: 27 - protein, 14 aa, synthetic construct
  REGION 1..14: note = 900725 HCDR3
ARYYGSDYEWYFDV

SEQ ID NO: 28 - protein, 8 aa, synthetic construct
  REGION 1..8: note = 900725 HCDR2
IHPNSGST

SEQ ID NO: 29 - protein, 8 aa, synthetic construct
  REGION 1..8: note = 900725 HCDR1
GYTFTSYW

SEQ ID NO: 30 - protein, 25 aa, synthetic construct
  REGION 1..25: note = 900725 H-FR1
QVQLVQSGAEVKKPGASVKLSCKAS

SEQ ID NO: 31 - protein, 17 aa, synthetic construct
  REGION 1..17: note = 900725 H-FR2
IHWVRQAPGQGLEWIGM

SEQ ID NO: 32 - protein, 38 aa, synthetic construct
  REGION 1..38: note = 900725 H-FR3
YYNEKFKGRATLTVDKSTSTAYMELSSLRSEDTAVYYC

SEQ ID NO: 33 - protein, 121 aa, synthetic construct
  REGION 1..121: note = 900725 VH
QVQLVQSGAEVKKPGASVKLSCKASGYTFTSYWIHWVRQAPGQGLEWIGMIHPNSGSTYYNEKFKGRATLTVDKSTSTAYMELSSLRSEDTAVYYCARYYGSDYEWYFDVWGQGTTVTVSS

SEQ ID NO: 34 - protein, 9 aa, synthetic construct
  REGION 1..9: note = 900725 LCDR3
LQHWNYPYT

SEQ ID NO: 35 - skipped

SEQ ID NO: 36 - protein, 6 aa, synthetic construct
  REGION 1..6: note = 900725 LCDR1
QNVRTA

SEQ ID NO: 37 - protein, 26 aa, synthetic construct
  REGION 1..26: note = 900725 L-FR1
DIQMTQSPSSMSASVGDRVTITCKAS

SEQ ID NO: 38 - protein, 17 aa, synthetic construct
  REGION 1..17: note = 900725 L-FR2
VVWYQQKPGKAPKALIY

SEQ ID NO: 39 - protein, 36 aa, synthetic construct
  REGION 1..36: note = 900725 L-FR3
NRHTGVPDRFSGSGSGTDFTLTISSLQPEDFATYFC

SEQ ID NO: 40 - protein, 107 aa, synthetic construct
  REGION 1..107: note = 900725 VL
DIQMTQSPSSMSASVGDRVTITCKASQNVRTAVVWYQQKPGKAPKALIYLASNRHTGVPDRFSGSGSGTDFTLTISSLQPEDFATYFCLQHWNYPYTFGQGTKLEIK

SEQ ID NO: 41 - protein, 450 aa, synthetic construct
  REGION 1..450: note = 900725 heavy chain
QVQLVQSGAEVKKPGASVKLSCKASGYTFTSYWIHWVRQAPGQGLEWIGMIHPNSGSTYYNEKFKGRATLTVDKSTSTAYMELSSLRSEDTAVYYCARYYGSDYEWYFDVWGQGTTVTVSSASTKGPSVFPLAPSSKSTSGGTAALGCLVKDYFPEPVTVSWNSGALTSGVHTFPAVLQSSGLYSLSSVVTVPSSSLGTQTYICNVNHKPSNTKVDKRVEPKSCDKTHTCPPCPAPEAAGGPSVFLFPPKPKDTLMISRTPEVTCVVVDVSHEDPEVKFNWYVDGVEVHNAKTKPREEQYNSTYRVVSVLTVLHQDWLNGKEYKCKVSNKALPAPIEKTISKAKGQPREPQVYTLPPSREEMTKNQVSLTCLVKGFYPSDIAVEWESNGQPENNYKTTPPVLDSDGSFFLYSKLTVDKSRWQQGNVFSCSVMHEALHNHYTQKSLSLSPG

SEQ ID NO: 42 - protein, 214 aa, synthetic construct
  REGION 1..214: note = 900725 light chain
DIQMTQSPSSMSASVGDRVTITCKASQNVRTAVVWYQQKPGKAPKALIYLASNRHTGVPDRFSGSGSGTDFTLTISSLQPEDFATYFCLQHWNYPYTFGQGTKLEIKRTVAAPSVFIFPPSDEQLKSGTASVVCLLNNFYPREAKVQWKVDNALQSGNSQESVTEQDSKDSTYSLSSTLTLSKADYEKHKVYACEVTHQGLSSPVTKSFNRGEC

SEQ ID NO: 43 - protein, 329 aa, synthetic construct
  REGION 1..329: note = heavy chain constant region
ASTKGPSVFPLAPSSKSTSGGTAALGCLVKDYFPEPVTVSWNSGALTSGVHTFPAVLQSSGLYSLSSVVTVPSSSLGTQTYICNVNHKPSNTKVDKRVEPKSCDKTHTCPPCPAPEAAGGPSVFLFPPKPKDTLMISRTPEVTCVVVDVSHEDPEVKFNWYVDGVEVHNAKTKPREEQYNSTYRVVSVLTVLHQDWLNGKEYKCKVSNKALPAPIEKTISKAKGQPREPQVYTLPPSREEMTKNQVSLTCLVKGFYPSDIAVEWESNGQPENNYKTTPPVLDSDGSFFLYSKLTVDKSRWQQGNVFSCSVMHEALHNHYTQKSLSLSPG

SEQ ID NO: 44 - protein, 107 aa, synthetic construct [sequence omitted]

SEQ ID NO: 45 - protein, 584 aa, synthetic construct
  REGION 1..584: note = 700035 heavy chain
QVQLVESGGGLVQPGGSLRLSCAASGSISSIAAMGWYRQAPGKERELVAAITSGGNTNLADSTKGRFTISRDNTKNTVYLQMNSLKPEDTAVYYCNAWGEDDSSWFGTDLCDYWGQGTQVTVSSGGGGSGGGGSQVQLVQSGAEVKKPGASVKLSCKASGYTFTSYWIHWVRQAPGQGLEWIGMIHPNSGSTYYNEKFKGRATLTVDKSTSTAYMELSSLRSEDTAVYYCARYYGSDYEWYFDVWGQGTTVTVSSASTKGPSVFPLAPSSKSTSGGTAALGCLVKDYFPEPVTVSWNSGALTSGVHTFPAVLQSSGLYSLSSVVTVPSSSLGTQTYICNVNHKPSNTKVDKRVEPKSCDKTHTCPPCPAPEAAGGPSVFLFPPKPKDTLMISRTPEVTCVVVDVSHEDPEVKFNWYVDGVEVHNAKTKPREEQYNSTYRVVSVLTVLHQDWLNGKEYKCKVSNKALPAPIEKTISKAKGQPREPQVYTLPPSREEMTKNQVSLTCLVKGFYPSDIAVEWESNGQPENNYKTTPPVLDSDGSFFLYSKLTVDKSRWQQGNVFSCSVMHEALHNHYTQKSLSLSPG

SEQ ID NO: 46 - protein, 588 aa, synthetic construct
  REGION 1..588: note = 700038 heavy chain
QVQLVESGGGLVQPGGSLRLSCAASGSISSIAAMGWYRQAPGKERELVAAITSGGNTNLADSTKGRFTISRDNTKNTVYLQMNSLKPEDTAVYYCNAWGEDDSSWFGTDLCDYWGQGTQVTVSSGGGGSGGGGSQVQLVESGGGLVKPGGSLRLSCAASGFTFSKYAMSWIRQAPGKGLEWVAEISSGGGYINYADSVKGRFTISRDNAKNSLYLQMNSLRAEDTAVYYCARAIYYYGSSYNYYAMDYWGQGTTVTVSSASTKGPSVFPLAPSSKSTSGGTAALGCLVKDYFPEPVTVSWNSGALTSGVHTFPAVLQSSGLYSLSSVVTVPSSSLGTQTYICNVNHKPSNTKVDKRVEPKSCDKTHTCPPCPAPEAAGGPSVFLFPPKPKDTLMISRTPEVTCVVVDVSHEDPEVKFNWYVDGVEVHNAKTKPREEQYNSTYRVVSVLTVLHQDWLNGKEYKCKVSNKALPAPIEKTISKAKGQPREPQVYTLPPSREEMTKNQVSLTCLVKGFYPSDIAVEWESNGQPENNYKTTPPVLDSDGSFFLYSKLTVDKSRWQQGNVFSCSVMHEALHNHYTQKSLSLSPG

SEQ ID NO: 47 - protein, 10 aa, synthetic construct
  REGION 1..10: note = linker
GGGGSGGGGS

SEQ ID NO: 48 - protein, 450 aa, synthetic construct
  REGION 1..450: note = 900543 heavy chain
QIQLVQSGPELKKPGETVKISCKTSGYTFTNYGMNWVKQAPGKGLKWVGWINTYTGEPKYADDFKGRFAFSVETSASTAYLQINNLKNEDTATYFCARGIYDGYHWYFDVWGAGTTVTVSSASTKGPSVFPLAPSSKSTSGGTAALGCLVKDYFPEPVTVSWNSGALTSGVHTFPAVLQSSGLYSLSSVVTVPSSSLGTQTYICNVNHKPSNTKVDKRVEPKSCDKTHTCPPCPAPEAAGGPSVFLFPPKPKDTLMISRTPEVTCVVVDVSHEDPEVKFNWYVDGVEVHNAKTKPREEQYNSTYRVVSVLTVLHQDWLNGKEYKCKVSNKALPAPIEKTISKAKGQPREPQVYTLPPSREEMTKNQVSLTCLVKGFYPSDIAVEWESNGQPENNYKTTPPVLDSDGSFFLYSKLTVDKSRWQQGNVFSCSVMHEALHNHYTQKSLSLSPG

SEQ ID NO: 49 - protein, 219 aa, synthetic construct
  REGION 1..219: note = 900543 light chain
DVVMTQTPLSLPVSLGDQASISCRSSQSLVHSIGNTYLHWYLQKPGQSPKLLIYKVSNRFSGVPDRFSGSGSGTDFTLKITRVEAEDLGVYFCSQSTHVPFTFGSGTKLEIKRTVAAPSVFIFPPSDEQLKSGTASVVCLLNNFYPREAKVQWKVDNALQSGNSQESVTEQDSKDSTYSLSSTLTLSKADYEKHKVYACEVTHQGLSSPVTKSFNRGEC